European Patent Application EP 4 763 223 A1, published June 24, 2026. Title: An engineered cell comprising a chimeric antigen receptor and a switchable chimeric antigen receptor, a kit and their use. Applicant: AvenCell Therapeutics Inc. Application EP. The sequence listing filed with the application follows.

SEQUENCE LISTING (102 sequences)

SEQ ID NO: 1 - protein, 8 aa, Mus musculus
GVSLPDYG

SEQ ID NO: 2 - protein, 7 aa, Mus musculus
IWGSETT

SEQ ID NO: 3 - protein, 14 aa, Mus musculus
AKHYYYGGSYAMDY

SEQ ID NO: 4 - protein, 6 aa, Mus musculus
QDISKY

SEQ ID NO: 5 - protein, 9 aa, Mus musculus
QQGNTLPYT

SEQ ID NO: 6 - protein, 245 aa, Mus musculus
DIQMTQTTSSLSASLGDRVTISCRASQDISKYLNWYQQKPDGTVKLLIYHTSRLHSGVPSRFSGSGSGTDYSLTISNLEQEDIATYFCQQGNTLPYTFGGGTKLEITGSTSGSGKPGSGEGSTKGEVKLQESGPGLVAPSQSLSVTCTVSGVSLPDYGVSWIRQPPRKGLEWLGVIWGSETTYYNSALKSRLTIIKDNSKSQVFLKMNSLQTDDTAIYYCAKHYYYGGSYAMDYWGQGTSVTVSS

SEQ ID NO: 7 - protein, 10 aa, Lama glama
GRTFSNYNMG

SEQ ID NO: 8 - protein, 18 aa, Lama glama
AIDWSGGSPYYAASVRGR

SEQ ID NO: 9 - protein, 12 aa, Lama glama
PLSYGSTWLADY

SEQ ID NO: 10 - protein, 121 aa, Lama glama
QVQLVESGGGLVQPGGSLRLSCAASGRTFSNYNMGWFRQAPGQGLEFVAAIDWSGGSPYYAASVRGRFTISRDNSKNTLYLQMNSLRAEDTAVYYCAAPLSYGSTWLADYWGQGTLVTVSS

SEQ ID NO: 11 - protein, 5 aa, synthetic construct
  source 1..5: note = linker sequence
GGGGS

SEQ ID NO: 12 - protein, 25 aa, synthetic construct
  source 1..25: note = linker sequence
GGGGSGGGGSGASAAGGGGSGGGGS

SEQ ID NO: 13 - protein, 25 aa, synthetic construct
  source 1..25: note = linker sequence
GGGGSGGGGSGGGGSGGGGSGGGGS

SEQ ID NO: 14 - protein, 18 aa, synthetic construct
  source 1..18: note = linker sequence
GSTSGSGKPGSGEGSTKG

SEQ ID NO: 15 - protein, 33 aa, Saccharomyces cerevisiae
RMKQLEPKVEELLPKNYHLENEVARLKKLVGER

SEQ ID NO: 16 - protein, 14 aa, Saccharomyces cerevisiae
NYHLENEVARLKKL

SEQ ID NO: 17 - protein, 51 aa, Homo sapiens
MDPDLEIRAAFLRQRNTALRTEVAELEQEVQRLENEVSQYETRYGPLGGGK

SEQ ID NO: 18 - protein, 51 aa, Homo sapiens
MDPDLEIEAAFLERENTALETRVAELRQRVQRLRNRVSQYRTRYGPLGGGK

SEQ ID NO: 19 - protein, 10 aa, Homo sapiens
KPLPEVTDEY

SEQ ID NO: 20 - protein, 20 aa, Homo sapiens
  VARIANT 16: note = Xaa can be alanine or serine
LEKEALKKIIEDQQEXLNKW

SEQ ID NO: 21 - protein, 20 aa, Homo sapiens
LEKEALKKIIEDQQEALNKW

SEQ ID NO: 22 - protein, 8 aa, synthetic construct
  source 1..8: note = Humanized CDR sequence
GYTFTHYY

SEQ ID NO: 23 - protein, 8 aa, Mus musculus
VNPSNGGT

SEQ ID NO: 24 - protein, 13 aa, synthetic construct
  source 1..13: note = Humanized CDR sequence
ARSEYDYGLGFAY

SEQ ID NO: 25 - protein, 12 aa, Mus musculus
QSLLNSRTPKNY

SEQ ID NO: 26 - protein, 8 aa, Mus musculus
KQSYNLLT

SEQ ID NO: 27 - protein, 113 aa, synthetic construct
  source 1..113: note = Humanized light chain of scFv
  VARIANT 24: note = Xaa can be any naturally occurring amino acid
  VARIANT 35: note = Xaa can be any naturally occurring amino acid
  VARIANT 61: note = Xaa can be any naturally occurring amino acid
  VARIANT 101: note = Xaa can be any naturally occurring amino acid
DIVMTQSPDSLAVSLGERATINCXSSQSLLNSRTXKNYLAWYQQKPGQPPKLLIYWASTRXSGVPDRFSGSGSGTDFTLTISSLQAEDVAVYYCKQSYNLXTFGGGTKVEILK

SEQ ID NO: 28 - protein, 112 aa, synthetic construct
  source 1..112: note = Humanized light chain of scFv
DIVMTQSPDSLAVSLGERATINCKSSQSLLNSRTPKNYLAWYQQKPGQPPKLLIYWASTRKSGVPDRFSGSGSGTDFTLTISSLQAEDVAVYYCKQSYNLLTFGGGTKVEIK

SEQ ID NO: 29 - protein, 120 aa, synthetic construct
  source 1..120: note = Humanized heavy chain of scFv
QVQLVQSGAEVKKPGASVKVSCKASGYTFTHYYIYWVRQAPGQGLEWMGGVNPSNGGTHFNEKFKSRVTMTRDTSISTAYMELSRLRSDDTAVYYCARSEYDYGLGFAYWGQGTLVTVSS

SEQ ID NO: 30 - protein, 112 aa, synthetic construct
  source 1..112: note = Humanized light chain of scFv
DIVMTQSPDSLAVSLGERATINCRSSQSLLDSRTKKNYLAWYQQKPGQPPKLLIYWASTRESGVPDRFSGSGSGTDFTLTISSLQAEDVAVYYCKQSYNLPTFGGGTKVEIK

SEQ ID NO: 31 - protein, 118 aa, synthetic construct
  source 1..118: note = Humanized heavy chain of scFv
EVQLVESGGGLVQPGGSLRLSCAASGFTFSDFWMNWVRQAPGKGLEWVGQIRNKPNNYETYYSDSLKGRFTISRDDSKSITYLQMNSLRAEDTAVYYCTLGNSWFAYWGQGTLVTVSS

SEQ ID NO: 32 - protein, 44 aa, Homo sapiens
TTTPAPRPPTPAPTIASQPLSLRPEACRPAAGGAVHTRGLDFAC

SEQ ID NO: 33 - protein, 54 aa, Homo sapiens
FVPVFLPAKPTTTPAPRPPTPAPTIASQPLSLRPEACRPAAGGAVHTRGLDFAC

SEQ ID NO: 34 - protein, 39 aa, Homo sapiens
IEVMYPPPYLDNEKSNGTIIHVKGKHLCPSPLFPGPSKP

SEQ ID NO: 35 - protein, 133 aa, synthetic construct
  source 1..133: note = CD28 extracellular hinge domain
KILVKQSPMLVAYDNAVNLSCKYSYNLFSREFRASLHKGLDSAVEVCVVYGNYSQQLQVYSKTGFNCDGKLGNESVTFYLQNLYVNQTDIYFCKIEVMAPPPALDNEKSNGTIIHVKGKHLCPSPLFPGPSKP

SEQ ID NO: 36 - protein, 12 aa, synthetic construct
  source 1..12: note = IgG4 extracellular hinge domain
ESKYGPPCPPCP

SEQ ID NO: 37 - protein, 15 aa, Homo sapiens
EPKSCDKTHTCPPCP

SEQ ID NO: 38 - protein, 12 aa, Homo sapiens
ERKCCVECPPCP

SEQ ID NO: 39 - protein, 25 aa, Homo sapiens
DIYIWAPLAGTCGVLLLSLVITLYC

SEQ ID NO: 40 - protein, 21 aa, Homo sapiens
IYIWAPLAGTCGVLLLSLVIT

SEQ ID NO: 41 - protein, 28 aa, Homo sapiens
MFWVLVVVGGVLACYSLLVTVAFIIFWV

SEQ ID NO: 42 - protein, 27 aa, Homo sapiens
FWVLVVVGGVLACYSLLVTVAFIIFWV

SEQ ID NO: 43 - protein, 21 aa, Homo sapiens
FWLPIGCAAFVVVCILGCILI

SEQ ID NO: 44 - protein, 22 aa, Homo sapiens
MALIVLGGVAGLLLFIGLGIFF

SEQ ID NO: 45 - protein, 112 aa, Homo sapiens
RVKFSRSADAPAYQQGQNQLYNELNLGRREEYDVLDKRRGRDPEMGGKPRRKNPQEGLYNELQKDKMAEAYSEIGMKGERRRGKGHDGLYQGLSTATKDTYDALHMQALPPR

SEQ ID NO: 46 - protein, 48 aa, Homo sapiens
QRRKYRSNKGESPVEPAEPCHYSCPREEEGSTIPIQEDYRKPEPACSP

SEQ ID NO: 47 - protein, 41 aa, Homo sapiens
RSKRSRLLHSDYMNMTPRRPGPTRKHYQPYAPPRDFAAYRS

SEQ ID NO: 48 - protein, 41 aa, synthetic construct
  source 1..41: note = CD28 intracellular signaling domain
RSKRSRGGHSDYMNMTPRRPGPTRKHYQPYAPPRDFAAYRS

SEQ ID NO: 49 - protein, 42 aa, Homo sapiens
ALYLLRRDQRLPPDAHKPPGGGSFRTPIQEEQADAHSTLAKI

SEQ ID NO: 50 - protein, 42 aa, Homo sapiens
KRGRKKLLYIFKQPFMRPVQTTQEEDGCSCRFPEEEEGGCEL

SEQ ID NO: 51 - protein, 42 aa, synthetic construct
  source 1..42: note = 4-1BB intracellular signaling domain
KRGRKKGGYIFKQPFMRPVQTTQEEDGCSCRFPEEEEGGCEL

SEQ ID NO: 52 - protein, 38 aa, Homo sapiens
CWLTKKKYSSSVHDPNGEYMFMRAVNTAKKSRLTDVTL

SEQ ID NO: 53 - protein, 24 aa, Homo sapiens
LCARPRRSPAQEDGKVYINMPGRG

SEQ ID NO: 54 - protein, 52 aa, Homo sapiens
YFLGRLVPRGRGAAEAATRKQRITETESPYQELQGQRSDVYSDLNTQRPYYK

SEQ ID NO: 55 - protein, 97 aa, Homo sapiens
CSRAARGTIGARRTGQPLKEDPSAVPVFSVDYGELDFQWREKTPEPPVPCVPEQTEYATIVFPSGMGTSSPARRGSADGPRSAQPLRPEDGHCSWPL

SEQ ID NO: 56 - protein, 41 aa, Homo sapiens
AVSLSKMLKKRSPLTTGVYVKMPPTEPECEKQFQPYFIPIN

SEQ ID NO: 57 - protein, 22 aa, Homo sapiens
MDMRVPAQLLGLLLLWLRGARC

SEQ ID NO: 58 - protein, 20 aa, synthetic construct
  source 1..20: note = signal peptide
MRRMQLLLLIALSLALVTNS

SEQ ID NO: 59 - protein, 21 aa, Homo sapiens
MKWKALFTAAILQAQLPITEA

SEQ ID NO: 60 - protein, 22 aa, Homo sapiens
MLLLVTSLLLCELPHPAFLLIP

SEQ ID NO: 61 - protein, 21 aa, Homo sapiens
MALPVTALLLPLALLLHAARP

SEQ ID NO: 62 - protein, 26 aa, synthetic construct
  source 1..26: note = cleavage site
RAKRSGSGEGRGSLLTCGDVEENPGP

SEQ ID NO: 63 - protein, 28 aa, synthetic construct
  source 1..28: note = cleavage site
GSGSSGEGRGSLLTCGDVEENPGPPVAT

SEQ ID NO: 64 - DNA, 241 bp, synthetic construct
  source 1..241: mol_type = other DNA; note = promoter
gggcagagcgcacatcgcccacagtccccgagaagttggggggaggggtcggcaattgaaccggtgcctagagaaggtggcgcggggtaaactgggaaagtgatgtcgtgtactggctccgcctttttcccgagggtgggggagaaccgtatataagtgcagtagtcgccgtgaacgttctttttcgcaacgggtttgccgccagaacacagctgaagctcgggatccaccggtcgccacc

SEQ ID NO: 65 - protein, 632 aa, synthetic construct
  source 1..632: note = chimeric antigen receptor
MALPVTALLLPLALLLHAARPQVQLVESGGGLVQPGGSLRLSCAASGRTFSNYNMGWFRQAPGQGLEFVAAIDWSGGSPYYAASVRGRFTISRDNSKNTLYLQMNSLRAEDTAVYYCAAPLSYGSTWLADYWGQGTLVTVSSGGGGSGGGGSGGGGSGGGGSGGGGSDIQMTQTTSSLSASLGDRVTISCRASQDISKYLNWYQQKPDGTVKLLIYHTSRLHSGVPSRFSGSGSGTDYSLTISNLEQEDIATYFCQQGNTLPYTFGGGTKLEITGSTSGSGKPGSGEGSTKGEVKLQESGPGLVAPSQSLSVTCTVSGVSLPDYGVSWIRQPPRKGLEWLGVIWGSETTYYNSALKSRLTIIKDNSKSQVFLKMNSLQTDDTAIYYCAKHYYYGGSYAMDYWGQGTSVTVSSIEVMYPPPYLDNEKSNGTIIHVKGKHLCPSPLFPGPSKPFWVLVVVGGVLACYSLLVTVAFIIFWVKRGRKKLLYIFKQPFMRPVQTTQEEDGCSCRFPEEEEGGCELRVKFSRSADAPAYQQGQNQLYNELNLGRREEYDVLDKRRGRDPEMGGKPRRKNPQEGLYNELQKDKMAEAYSEIGMKGERRRGKGHDGLYQGLSTATKDTYDALHMQALPPR

SEQ ID NO: 66 - protein, 631 aa, synthetic construct
  source 1..631: note = chimeric antigen receptor
MALPVTALLLPLALLLHAARPQVQLVESGGGLVQPGGSLRLSCAASGRTFSNYNMGWFRQAPGQGLEFVAAIDWSGGSPYYAASVRGRFTISRDNSKNTLYLQMNSLRAEDTAVYYCAAPLSYGSTWLADYWGQGTLVTVSSGGGGSGGGGSGGGGSGGGGSGGGGSDIQMTQTTSSLSASLGDRVTISCRASQDISKYLNWYQQKPDGTVKLLIYHTSRLHSGVPSRFSGSGSGTDYSLTISNLEQEDIATYFCQQGNTLPYTFGGGTKLEITGSTSGSGKPGSGEGSTKGEVKLQESGPGLVAPSQSLSVTCTVSGVSLPDYGVSWIRQPPRKGLEWLGVIWGSETTYYNSALKSRLTIIKDNSKSQVFLKMNSLQTDDTAIYYCAKHYYYGGSYAMDYWGQGTSVTVSSIEVMYPPPYLDNEKSNGTIIHVKGKHLCPSPLFPGPSKPFWVLVVVGGVLACYSLLVTVAFIIFWVRSKRSRLLHSDYMNMTPRRPGPTRKHYQPYAPPRDFAAYRSRVKFSRSADAPAYQQGQNQLYNELNLGRREEYDVLDKRRGRDPEMGGKPRRKNPQEGLYNELQKDKMAEAYSEIGMKGERRRGKGHDGLYQGLSTATKDTYDALHMQALPPR

SEQ ID NO: 67 - protein, 634 aa, synthetic construct
  source 1..634: note = chimeric antigen receptor
MALPVTALLLPLALLLHAARPQVQLVESGGGLVQPGGSLRLSCAASGRTFSNYNMGWFRQAPGQGLEFVAAIDWSGGSPYYAASVRGRFTISRDNSKNTLYLQMNSLRAEDTAVYYCAAPLSYGSTWLADYWGQGTLVTVSSGGGGSGGGGSGGGGSGGGGSGGGGSDIQMTQTTSSLSASLGDRVTISCRASQDISKYLNWYQQKPDGTVKLLIYHTSRLHSGVPSRFSGSGSGTDYSLTISNLEQEDIATYFCQQGNTLPYTFGGGTKLEITGSTSGSGKPGSGEGSTKGEVKLQESGPGLVAPSQSLSVTCTVSGVSLPDYGVSWIRQPPRKGLEWLGVIWGSETTYYNSALKSRLTIIKDNSKSQVFLKMNSLQTDDTAIYYCAKHYYYGGSYAMDYWGQGTSVTVSSAAAIEVMYPPPYLDNEKSNGTIIHVKGKHLCPSPLFPGPSKPFWVLVVVGGVLACYSLLVTVAFIIFWVRSKRSRLLHSDYMNMTPRRPGPTRKHYQPYAPPRDFAAYRSRVKFSRSADAPAYQQGQNQLYNELNLGRREEYDVLDKRRGRDPEMGGKPRRKNPQEGLYNELQKDKMAEAYSEIGMKGERRRGKGHDGLYQGLSTATKDTYDALHMQALPPR

SEQ ID NO: 68 - DNA, 1896 bp, synthetic construct
  source 1..1896: mol_type = other DNA; note = chimeric antigen receptor
atggcccttccagtgaccgccctgctgctgccactggctctgctgctgcacgccgctagacctcaggtgcagctggtggaaagcggcgggggcctggtgcagcctggcggcagcctgagactgtcttgcgccgctagcggaagaacttttagcaactacaacatgggctggtttagacaggcccccggccagggcctggagttcgtggctgccatcgactggagcggcggaagcccctattacgccgcctccgtgcggggcagattcaccatcagccgggacaattctaagaataccctgtatctgcaaatgaacagcctgagagccgaagatacagccgtgtactactgcgccgcccctctgagctacggaagcacatggctggccgactactggggacaaggaaccctggtaaccgtctcaagcggcggtggaggatcaggaggtggtggttcaggaggtggaggttctgggggaggcggatctgggggaggaggcagcgacatccagatgacacagacaacctccagcctgagcgccagcctgggcgacagagtgaccatcagctgtagagcctctcaggacatcagcaagtacctgaactggtatcagcagaaacctgatggcaccgtgaagctgctgatctaccacacatctaggctgcactctggagtccccagccggtttagcggaagcgggtcaggcacagactatagcctgaccatctccaatctggaacaggaggacatcgccacctacttctgccagcagggcaacaccctgccttatacattcggtggcggcaccaagctggaaatcaccggcagcacctctggctctggcaagcccggaagcggcgagggctccaccaagggagaggtgaagctgcaggagtccggacctgggctggtggctccaagccagagcctgagcgtgacctgcaccgtgtccggagtgagcctgcctgattacggcgtgtcttggatcagacagcctcctagaaagggactggaatggctgggcgtgatctggggtagcgagacaacatactacaacagcgccctgaagagcagactgacaatcatcaaggacaacagcaaaagccaggtgttcctaaaaatgaactccctgcagaccgacgacaccgccatctactactgtgcgaaacactactactacggcggctcctacgccatggactattggggccagggcaccagcgtgacagtgagcagcatcgaggtgatgtacccccctccttacctggacaacgagaagtccaacggcaccattatccacgtgaaaggcaagcacctgtgccccagccctctgttccccggcccttctaaaccgttctgggttctggtggtcgtgggcggcgtactggcttgctactctctgctggtcacagtggctttcatcatcttctgggtgaaaagaggcagaaagaaactgctgtacatctttaagcagccattcatgcggccagtgcagaccacccaggaggaggacggctgctcttgtcgctttcccgaggaggaggagggcggatgtgagctgagggtgaagtttagcagatccgctgatgcccctgcctatcagcagggacagaaccagctgtacaacgagctgaacctggggagaagagaagagtacgatgtgctggacaagcggagaggcagagatcctgagatgggcggcaagcccagacggaagaatcctcaagagggcctgtacaatgaactgcagaaagacaagatggccgaggcctacagcgagatcggaatgaagggcgagcgcagaagaggcaagggacacgatggactgtaccagggcctgagcaccgccaccaaggatacctatgatgccctgcacatgcaggccctgcctccaaga

SEQ ID NO: 69 - DNA, 1899 bp, synthetic construct
  source 1..1899: mol_type = other DNA; note = chimeric antigen receptor
atggccctgccagtgaccgccctgctgctgcccctggcactgctgctgcacgcagccagaccccaagtgcagctggtggagtcaggcggcgggctagtgcagccaggaggctccctgagactgtcttgcgctgcaagcggcagaaccttctcaaactacaatatggggtggttcaggcaggcccccgggcagggcctggagttcgtggccgctatcgactggagtgggggctccccctactatgcagctagcgtgagaggcagatttaccatctccagagacaactccaagaacactctgtacctccagatgaatagtctgagagccgaagatacagccgtgtactactgtgccgcccccctgagctacggcagcacctggctggctgattactggggtcagggaacactggttacagtgtcatccggaggaggtggtagtggaggcggaggcagtggtggaggcggtagcgggggaggcggatctgggggaggaggcagcgacatccagatgacccagaccacctcctctctgagcgcttcactcggagaccgggtgacaatcagctgtagagcctcccaggatatctctaagtatctgaactggtaccagcagaagccagatggcacagtgaagctgctgatctatcataccagcaggctgcactccggagtgccttccaggttttccggcagcggatccggcaccgattatagcctgaccatctccaatctggagcaggaggacatagcaacctacttttgccagcagggcaataccctgccctacacctttgggggaggaaccaaactcgaaatcaccggctctacttctggaagcggcaagcccggatcaggcgaaggctcaaccaagggcgaggtgaaactgcaggagagcggcccaggactggtcgccccatcacagtccctgtcagtgacctgcaccgttagcggggtgtccctgcctgactacggggtgagctggatcaggcagcctcctcggaagggcctggagtggctgggggtgatctggggctccgagaccacctattataactccgccctgaagtcccggctgaccatcattaaagataacagcaagagccaggtgttcctgaagatgaactcactgcagacagacgacaccgctatctattattgcgccaagcattactactacggcggatcatacgccatggactattggggccagggcacttctgtgaccgtgtcttctatcgaggtgatgtaccccccaccatatctggataacgagaaatccaatggcaccatcattcacgtgaagggcaagcacctgtgtccatctcctctgttccctggcccaagcaagcccttctgggtgctggtggtcgtggggggcgtgctggcctgctactctctgctggtgactgtggcattcatcatcttctgggtgaagcggggcaggaagaaactgctgtacatcttcaagcagccattcatgcggcccgtgcagaccacccaggaagaggatgggtgctcatgccggttccctgaggaggaggagggggggtgcgagctgagggtcaagttttccagaagcgctgacgctcccgcttaccagcagggccaaaatcagctctataacgaactgaatctcggcaggcgcgaggaatatgacgtgctggataagaggcggggacgcgaccctgaaatgggaggaaagcctcggcggaaaaacccacaagaaggactttacaacgaactccaaaaggataagatggctgaagcctactctgagattggcatgaaaggagaacgtcggagaggaaaaggccacgacggactctatcagggactgtctacagccacaaaagacacatacgacgcactccatatgcaggctctcccacctagataa

SEQ ID NO: 70 - DNA, 1893 bp, synthetic construct
  source 1..1893: mol_type = other DNA; note = chimeric antigen receptor
atggccctgccagtgaccgccctgctgctgcccctggcactgctgctgcacgcagccagaccccaagtgcagctggtggagtcaggcggcgggctagtgcagccaggaggctccctgagactgtcttgcgctgcaagcggcagaaccttctcaaactacaatatggggtggttcaggcaggcccccgggcagggcctggagttcgtggccgctatcgactggagtgggggctccccctactatgcagctagcgtgagaggcagatttaccatctccagagacaactccaagaacactctgtacctccagatgaatagtctgagagccgaagatacagccgtgtactactgtgccgcccccctgagctacggcagcacctggctggctgattactggggacagggtacactggttacagtatcatctggcggtggaggatcaggaggtggtggttcaggaggtggaggttctgggggaggcggatctgggggaggaggcagcgacatccagatgacccagaccacctcctctctgagcgcttcactcggagaccgggtgacaatcagctgtagagcctcccaggatatctctaagtatctgaactggtaccagcagaagccagatggcacagtgaagctgctgatctatcataccagcaggctgcactccggagtgccttccaggttttccggcagcggatccggcaccgattatagcctgaccatctccaatctggagcaggaggacatagcaacctacttttgccagcagggcaataccctgccctacacctttgggggaggaaccaaactcgaaatcaccggctctacttctggaagcggcaagcccggatcaggcgaaggctcaaccaagggcgaggtgaaactgcaggagagcggcccaggactggtcgccccatcacagtccctgtcagtgacctgcaccgttagcggggtgtccctgcctgactacggggtgagctggatcaggcagcctcctcggaagggcctggagtggctgggggtgatctggggctccgagaccacctattataactccgccctgaagtcccggctgaccatcattaaagataacagcaagagccaggtgttcctgaagatgaactcactgcagacagacgacaccgctatctattattgcgccaagcattactactacggcggatcatacgccatggactattggggccagggcacttctgtgaccgtgtcttctatcgaggtgatgtaccccccaccatatctggataacgagaaatccaatggcaccatcattcacgtgaagggcaagcacctgtgtccatctcctctgttccctggcccaagcaagcccttctgggtgctggtggtcgtggggggcgtgctggcctgctactctctgctggtgactgtggcattcatcatcttctgggtgagatccaaaaggtctcgcctgctgcacagcgactatatgaatatgacccctcgcaggcctggccctacacgcaagcactatcagccttacgccccccctcgggactttgctgcgtatcggagtagggtgaagtttagcagatccgctgatgcccctgcctatcagcagggacagaaccagctgtacaacgagctgaacctggggagaagagaagagtacgatgtgctggacaagcggagaggcagagatcctgagatgggcggcaagcccagacggaagaatcctcaagagggcctgtacaatgaactgcagaaagacaagatggccgaggcctacagcgagatcggaatgaagggcgagcgcagaagaggcaagggacacgatggactgtaccagggcctgagcaccgccaccaaggatacctatgatgccctgcacatgcaggccctgcctccaaga

SEQ ID NO: 71 - DNA, 1896 bp, synthetic construct
  source 1..1896: mol_type = other DNA; note = chimeric antigen receptor
atggccctgccagtgaccgccctgctgctgcccctggcactgctgctgcacgcagccagaccccaagtgcagctggtggagtcaggcggcgggctagtgcagccaggaggctccctgagactgtcttgcgctgcaagcggcagaaccttctcaaactacaatatggggtggttcaggcaggcccccgggcagggcctggagttcgtggccgctatcgactggagtgggggctccccctactatgcagctagcgtgagaggcagatttaccatctccagagacaactccaagaacactctgtacctccagatgaatagtctgagagccgaagatacagccgtgtactactgtgccgcccccctgagctacggcagcacctggctggctgattactggggacagggtacactggttacagtatcatctggcggtggaggatcaggaggtggtggttcaggaggtggaggttctgggggaggcggatctgggggaggaggcagcgacatccagatgacccagaccacctcctctctgagcgcttcactcggagaccgggtgacaatcagctgtagagcctcccaggatatctctaagtatctgaactggtaccagcagaagccagatggcacagtgaagctgctgatctatcataccagcaggctgcactccggagtgccttccaggttttccggcagcggatccggcaccgattatagcctgaccatctccaatctggagcaggaggacatagcaacctacttttgccagcagggcaataccctgccctacacctttgggggaggaaccaaactcgaaatcaccggctctacttctggaagcggcaagcccggatcaggcgaaggctcaaccaagggcgaggtgaaactgcaggagagcggcccaggactggtcgccccatcacagtccctgtcagtgacctgcaccgttagcggggtgtccctgcctgactacggggtgagctggatcaggcagcctcctcggaagggcctggagtggctgggggtgatctggggctccgagaccacctattataactccgccctgaagtcccggctgaccatcattaaagataacagcaagagccaggtgttcctgaagatgaactcactgcagacagacgacaccgctatctattattgcgccaagcattactactacggcggatcatacgccatggactattggggccagggcacttctgtgaccgtgtcttctatcgaggtgatgtaccccccaccatatctggataacgagaaatccaatggcaccatcattcacgtgaagggcaagcacctgtgtccatctcctctgttccctggcccaagcaagcccttctgggtgctggtggtcgtggggggcgtgctggcctgctactctctgctggtgactgtggcattcatcatcttctgggtgagatccaaaaggtctcgcctgctgcacagcgactatatgaatatgacccctcgcaggcctggccctacacgcaagcactatcagccttacgccccccctcgggactttgctgcgtatcggagtagggtcaagttttccagaagcgctgacgctcccgcttaccagcagggccaaaatcagctctataacgaactgaatctcggcaggcgcgaggaatatgacgtgctggataagaggcggggacgcgaccctgaaatgggaggaaagcctcggcggaaaaacccacaagaaggactttacaacgaactccaaaaggataagatggctgaagcctactctgagattggcatgaaaggagaacgtcggagaggaaaaggccacgacggactctatcagggactgtctacagccacaaaagacacatacgacgcactccatatgcaggctctcccacctagataa

SEQ ID NO: 72 - DNA, 1902 bp, synthetic construct
  source 1..1902: mol_type = other DNA; note = chimeric antigen receptor
atggcccttccagtgaccgccctgctgctgccactggctctgctgctgcacgccgctagacctcaggtgcagctggtggaaagcgggggaggcctggttcagcccggcggcagcctgagactgagctgcgccgctagcggcagaacattcagcaactacaacatgggctggttcagacaagcccctggccagggcctggaattcgtggccgctatcgactggtccggcggcagcccttactacgccgcctccgtgcggggcagattcaccatctctcgggataatagcaagaacaccctctacctgcagatgaatagcctgagagccgaggataccgccgtgtactactgtgccgctcctctgtcttacggcagcacctggctggcagattactggggccagggcaccctggtgacagtgtccagcggcggaggaggcagcggcggaggcggaagcggcggtggtggctctggaggcggcggctccggcggtggcggcagtgatatccagatgacccagaccacttccagcctgtctgcctccctgggcgacagggtgactatcagctgccgcgccagccaggatatttcaaaatacctgaattggtaccagcagaagcccgacggcacagtgaagctgctgatctaccacaccagtcgcctgcacagcggcgtgcccagcaggttcagcggcagcggatccggcacagactacagcctgaccatcagcaacctggagcaggaggatatcgcaacttatttttgccagcagggcaatacactgccttacaccttcggcggcggcaccaagctggaaatcaccggcagcacaagtggctccggcaaaccaggcagcggagagggcagcacaaagggcgaggtgaaactgcaggagagcggccccggcctggtggcccccagccagtctctgagcgtgacctgcaccgtgtccggcgtgtccctgcctgactacggggtgagctggatcaggcagccccccaggaaaggcttggaatggctgggcgtgatctggggcagcgagacaacctattataactctgccctgaagagcagactgaccatcatcaaagacaatagcaaaagccaggtgttcctgaagatgaattcactgcagactgacgatactgccatctattattgtgccaaacactactactatggcggatcctatgccatggattactggggccagggcacctcagtgaccgtgtcctcggccgctgctattgaagtgatgtatccacccccttacctggacaacgagaaatcaaacggcactattatccacgtgaagggaaagcacctgtgcccctcccctctgtttcccggcccaagtaagcccttttgggtgctggtggtggtcgggggcgtgctggcctgttattccctgctggtcacagtggctttcatcatcttctgggtgcgcagcaagaggtccagactgctgcactctgactacatgaacatgactcccaggaggccaggccctactagaaaacactaccagccctacgctcctcctagagacttcgccgcctacaggtccagggtcaagttttccagaagcgctgacgctcccgcttaccagcagggccaaaatcagctctataacgaactgaatctcggcaggcgcgaggaatatgacgtgctggataagaggcggggacgcgaccctgaaatgggaggaaagcctcggcggaaaaacccacaagaaggactttacaacgaactccaaaaggataagatggctgaagcctactctgagattggcatgaaaggagaacgtcggagaggaaaaggccacgacggactctatcagggactgtctacagccacaaaagacacatacgacgcactccatatgcaggctctcccacctaga

SEQ ID NO: 73 - DNA, 1893 bp, synthetic construct
  source 1..1893: mol_type = other DNA; note = chimeric antigen receptor
atggcccttccagtgaccgccctgctgctgccactggctctgctgctgcacgccgctagacctcaggtgcagctggtggaaagcgggggaggcctggttcagcccggcggcagcctgagactgagctgcgccgctagcggcagaacattcagcaactacaacatgggctggttcagacaagcccctggccagggcctggaattcgtggccgctatcgactggtccggcggcagcccttactacgccgcctccgtgcggggcagattcaccatctctcgggataatagcaagaacaccctctacctgcagatgaatagcctgagagccgaggataccgccgtgtactactgtgccgctcctctgtcttacggcagcacctggctggcagattactggggccagggcaccctggtgacagtgtccagcggcggaggaggcagcggcggaggcggaagcggcggtggtggctctggaggcggcggctccggcggtggcggcagtgatatccagatgacccagaccacttccagcctgtctgcctccctgggcgacagggtgactatcagctgccgcgccagccaggatatttcaaaatacctgaattggtaccagcagaagcccgacggcacagtgaagctgctgatctaccacaccagtcgcctgcacagcggcgtgcccagcaggttcagcggcagcggatccggcacagactacagcctgaccatcagcaacctggagcaggaggatatcgcaacttatttttgccagcagggcaatacactgccttacaccttcggcggcggcaccaagctggaaatcaccggcagcacaagtggctccggcaaaccaggcagcggagagggcagcacaaagggcgaggtgaaactgcaggagagcggccccggcctggtggcccccagccagtctctgagcgtgacctgcaccgtgtccggcgtgtccctgcctgactacggggtgagctggatcaggcagccccccaggaaaggcttggaatggctgggcgtgatctggggcagcgagacaacctattataactctgccctgaagagcagactgaccatcatcaaagacaatagcaaaagccaggtgttcctgaagatgaattcactgcagactgacgatactgccatctattattgtgccaaacactactactatggcggatcctatgccatggattactggggccagggcacctcagtgaccgtgtcctcgattgaagtgatgtatccacccccttacctggacaacgagaaatcaaacggcactattatccacgtgaagggaaagcacctgtgcccctcccctctgtttcccggcccaagtaagcccttttgggtgctggtggtggtcgggggcgtgctggcctgttattccctgctggtcacagtggctttcatcatcttctgggtgcgcagcaagaggtccagactgctgcactctgactacatgaacatgactcccaggaggccaggccctactagaaaacactaccagccctacgctcctcctagagacttcgccgcctacaggtccagggtcaagttttccagaagcgctgacgctcccgcttaccagcagggccaaaatcagctctataacgaactgaatctcggcaggcgcgaggaatatgacgtgctggataagaggcggggacgcgaccctgaaatgggaggaaagcctcggcggaaaaacccacaagaaggactttacaacgaactccaaaaggataagatggctgaagcctactctgagattggcatgaaaggagaacgtcggagaggaaaaggccacgacggactctatcagggactgtctacagccacaaaagacacatacgacgcactccatatgcaggctctcccacctaga

SEQ ID NO: 74 - protein, 230 aa, synthetic construct
  source 1..230: note = switchable chimeric antigen receptor
MDMRVPAQLLGLLLLWLRGARCEFKPLPEVTDEYAAAESKYGPPCPPCPMFWVLVVVGGVLACYSLLVTVAFIIFWVRSKRSRLLHSDYMNMTPRRPGPTRKHYQPYAPPRDFAAYRSRVKFSRSADAPAYQQGQNQLYNELNLGRREEYDVLDKRRGRDPEMGGKPRRKNPQEGLYNELQKDKMAEAYSEIGMKGERRRGKGHDGLYQGLSTATKDTYDALHMQALPPR

SEQ ID NO: 75 - protein, 227 aa, synthetic construct
  source 1..227: note = switchable chimeric antigen receptor
MDMRVPAQLLGLLLLWLRGARCEFKPLPEVTDEYAAAESKYGPPCPPCPDIYIWAPLAGTCGVLLLSLVITLYCRSKRSRLLHSDYMNMTPRRPGPTRKHYQPYAPPRDFAAYRSRVKFSRSADAPAYQQGQNQLYNELNLGRREEYDVLDKRRGRDPEMGGKPRRKNPQEGLYNELQKDKMAEAYSEIGMKGERRRGKGHDGLYQGLSTATKDTYDALHMQALPPR

SEQ ID NO: 76 - protein, 231 aa, synthetic construct
  source 1..231: note = switchable chimeric antigen receptor
MDMRVPAQLLGLLLLWLRGARCEFKPLPEVTDEYAAAESKYGPPCPPCPMFWVLVVVGGVLACYSLLVTVAFIIFWVKRGRKKLLYIFKQPFMRPVQTTQEEDGCSCRFPEEEEGGCELRVKFSRSADAPAYQQGQNQLYNELNLGRREEYDVLDKRRGRDPEMGGKPRRKNPQEGLYNELQKDKMAEAYSEIGMKGERRRGKGHDGLYQGLSTATKDTYDALHMQALPPR

SEQ ID NO: 77 - protein, 257 aa, synthetic construct
  source 1..257: note = switchable chimeric antigen receptor
MDMRVPAQLLGLLLLWLRGARCEFKPLPEVTDEYAAAIEVMYPPPYLDNEKSNGTIIHVKGKHLCPSPLFPGPSKPFWVLVVVGGVLACYSLLVTVAFIIFWVKRGRKKLLYIFKQPFMRPVQTTQEEDGCSCRFPEEEEGGCELRVKFSRSADAPAYQQGQNQLYNELNLGRREEYDVLDKRRGRDPEMGGKPRRKNPQEGLYNELQKDKMAEAYSEIGMKGERRRGKGHDGLYQGLSTATKDTYDALHMQALPPR

SEQ ID NO: 78 - protein, 255 aa, synthetic construct
  source 1..255: note = switchable chimeric antigen receptor
MDMRVPAQLLGLLLLWLRGARCEFKPLPEVTDEYDIEVMYPPPYLDNEKSNGTIIHVKGKHLCPSPLFPGPSKPFWVLVVVGGVLACYSLLVTVAFIIFWVKRGRKKLLYIFKQPFMRPVQTTQEEDGCSCRFPEEEEGGCELRVKFSRSADAPAYQQGQNQLYNELNLGRREEYDVLDKRRGRDPEMGGKPRRKNPQEGLYNELQKDKMAEAYSEIGMKGERRRGKGHDGLYQGLSTATKDTYDALHMQALPPR

SEQ ID NO: 79 - protein, 227 aa, synthetic construct
  source 1..227: note = switchable chimeric antigen receptor
MDMRVPAQLLGLLLLWLRGARCEFKPLPEVTDEYAAAESKYGPPCPPCPIYIWAPLAGTCGVLLLSLVITLYCKRGRKKLLYIFKQPFMRPVQTTQEEDGCSCRFPEEEEGGCELRVKFSRSADAPAYQQGQNQLYNELNLGRREEYDVLDKRRGRDPEMGGKPRRKNPQEGLYNELQKDKMAEAYSEIGMKGERRRGKGHDGLYQGLSTATKDTYDALHMQALPPR

SEQ ID NO: 80 - DNA, 693 bp, synthetic construct
  source 1..693: mol_type = other DNA; note = switchable chimeric antigen receptor
atggacatgagagtgccagctcagctgctgggcctgctgctgctgtggctgagaggcgccagatgcgagttcaagcctctgcctgaagtgaccgacgagtacgccgccgctgagtctaagtacggccctccttgtcctccttgccctatgttttgggtgctggttgtggttggaggcgtgctcgcttgttactccctcctggtgacagtcgcttttatcattttttgggtgcgcagcaagaggtccagactgctgcactctgactacatgaacatgactcccaggaggccaggccctactagaaaacactaccagccctacgctcctcctagagacttcgccgcctacaggtccagggtcaagttttccagaagcgctgacgctcccgcttaccagcagggccaaaatcagctctataacgaactgaatctcggcaggcgcgaggaatatgacgtgctggataagaggcggggacgcgaccctgaaatgggaggaaagcctcggcggaaaaacccacaagaaggactttacaacgaactccaaaaggataagatggctgaagcctactctgagattggcatgaaaggagaacgtcggagaggaaaaggccacgacggactctatcagggactgtctacagccacaaaagacacatacgacgcactccatatgcaggctctcccacctagataa

SEQ ID NO: 81 - DNA, 681 bp, synthetic construct
  source 1..681: mol_type = other DNA; note = switchable chimeric antigen receptor
atggatatgagggtgccagcccagctgctgggcctgctgctgctgtggctgagaggagccaggtgtgaatttaagcccctgcctgaggtgactgacgagtacgccgcagctgagtccaagtacggcccaccctgcccaccctgcccagacatctacatttgggcccctctggccggaacatgcggagtgctgcttctgtcccttgtaatcaccctttattgtcgatccaagagatcacgactgctgcattctgattacatgaatatgactcctagacggccagggcccacaaggaagcactaccagccttatgcccctcctagagatttcgccgcctatagaagtagggtgaagtttagcagatccgctgatgcccctgcctatcagcagggacagaaccagctgtacaacgagctgaacctggggagaagagaagagtacgatgtgctggacaagcggagaggcagagatcctgagatgggcggcaagcccagacggaagaatcctcaagagggcctgtacaatgaactgcagaaagacaagatggccgaggcctacagcgagatcggaatgaagggcgagcgcagaagaggcaagggacacgatggactgtaccagggcctgagcaccgccaccaaggatacctatgatgccctgcacatgcaggcactgcctccaaga

SEQ ID NO: 82 - DNA, 696 bp, synthetic construct
  source 1..696: mol_type = other DNA; note = switchable chimeric antigen receptor
atggacatgagagtgccagctcagctgctgggcctgctgctgctgtggctgagaggcgccagatgcgagttcaagcctctgcctgaagtgaccgacgagtacgccgccgctgagtctaagtacggccctccttgtcctccttgccctatgttttgggtcctggttgtggttggaggcgtgctcgcttgttactccctcctggtgacagtcgcttttatcattttttgggtgaagaggggccgcaagaagctgctgtatatctttaagcagccatttatgcggcccgtgcagaccacccaagaagaggacggatgtagctgcagatttcctgaggaagaagagggcggctgtgaactgagggtcaagttttccagaagcgctgacgctcccgcttaccagcagggccaaaatcagctctataacgaactgaatctcggcaggcgcgaggaatatgacgtgctggataagaggcggggacgcgaccctgaaatgggaggaaagcctcggcggaaaaacccacaagaaggactttacaacgaactccaaaaggataagatggctgaagcctactctgagattggcatgaaaggagaacgtcggagaggaaaaggccacgacggactctatcagggactgtctacagccacaaaagacacatacgacgcactccatatgcaggctctcccacctagataa

SEQ ID NO: 83 - DNA, 774 bp, synthetic construct
  source 1..774: mol_type = other DNA; note = switchable chimeric antigen receptor
atggacatgagagtgccagctcagctgctgggcctgctgctgctgtggctgagaggcgccagatgcgagttcaagcctctgcctgaagtgaccgacgagtacgccgccgctattgaagtcatgtatccacctccctatctggacaatgaaaagtctaatggcacaatcatccacgtcaagggaaaacacctgtgccctagccccctgtttcctggcccctctaaacccttttgggtcctggttgtggttggaggcgtgctcgcttgttactccctcctggtgacagtcgcttttatcattttttgggtgaagaggggccgcaagaagctgctgtatatctttaagcagccatttatgcggcccgtgcagaccacccaagaagaggacggatgtagctgcagatttcctgaggaagaagagggcggctgtgaactgagggtcaagttttccagaagcgctgacgctcccgcttaccagcagggccaaaatcagctctataacgaactgaatctcggcaggcgcgaggaatatgacgtgctggataagaggcggggacgcgaccctgaaatgggaggaaagcctcggcggaaaaacccacaagaaggactttacaacgaactccaaaaggataagatggctgaagcctactctgagattggcatgaaaggagaacgtcggagaggaaaaggccacgacggactctatcagggactgtctacagccacaaaagacacatacgacgcactccatatgcaggctctcccacctagataa

SEQ ID NO: 84 - DNA, 768 bp, synthetic construct
  source 1..768: mol_type = other DNA; note = switchable chimeric antigen receptor
atggatatgagagtgccagcccagctgctgggcctgctgctgctgtggctgagaggcgccagatgcgagttcaagcctctgccagaggtgactgatgagtacgacatcgaggtgatgtacccccctccttacctggacaacgagaagtccaacggcaccattatccacgtgaaaggcaagcacctgtgccccagccctctgttccccggcccttctaaaccgttctgggttctggtggtcgtgggcggcgtactggcttgctactctctgctggtcacagtggctttcatcatcttctgggtgaaaagaggcagaaagaaactgctgtacatctttaagcagccattcatgcggccagtgcagaccacccaggaggaggacggctgctcttgtcgctttcccgaggaggaggagggcggatgtgagctgagggtgaagtttagcagatccgctgatgcccctgcctatcagcagggacagaaccagctgtacaacgagctgaacctggggagaagagaagagtacgatgtgctggacaagcggagaggcagagatcctgagatgggcggcaagcccagacggaagaatcctcaagagggcctgtacaatgaactgcagaaagacaagatggccgaggcctacagcgagatcggaatgaagggcgagcgcagaagaggcaagggacacgatggactgtaccagggcctgagcaccgccaccaaggatacctatgatgccctgcacatgcaggccctgcctccaagataa

SEQ ID NO: 85 - DNA, 684 bp, synthetic construct
  source 1..684: mol_type = other DNA; note = switchable chimeric antigen receptor
atggatatgagagtgccagcccagctgctgggcctgctgctgctgtggctgagaggcgccagatgcgagttcaagcctctgccagaggtgactgatgagtacgcagccgctgaatcaaagtacggccctccttgtccaccctgtccaatctacatttgggcccccctggccgggacatgcggcgtgctcctgctgtctctggtgatcaccctgtactgtaaaagaggcagaaagaaactgctgtacatctttaagcagccattcatgcggccagtgcagaccacccaggaggaggacggctgctcttgtcgctttcccgaggaggaggagggcggatgtgagctgagggtgaagtttagcagatccgctgatgcccctgcctatcagcagggacagaaccagctgtacaacgagctgaacctggggagaagagaagagtacgatgtgctggacaagcggagaggcagagatcctgagatgggcggcaagcccagacggaagaatcctcaagagggcctgtacaatgaactgcagaaagacaagatggccgaggcctacagcgagatcggaatgaagggcgagcgcagaagaggcaagggacacgatggactgtaccagggcctgagcaccgccaccaaggatacctatgatgccctgcacatgcaggccctgcctccaagataa

SEQ ID NO: 86 - protein, 888 aa, synthetic construct
  source 1..888: note = chimeric antigen receptor and switchable chimeric antigen receptor
MALPVTALLLPLALLLHAARPQVQLVESGGGLVQPGGSLRLSCAASGRTFSNYNMGWFRQAPGQGLEFVAAIDWSGGSPYYAASVRGRFTISRDNSKNTLYLQMNSLRAEDTAVYYCAAPLSYGSTWLADYWGQGTLVTVSSGGGGSGGGGSGGGGSGGGGSGGGGSDIQMTQTTSSLSASLGDRVTISCRASQDISKYLNWYQQKPDGTVKLLIYHTSRLHSGVPSRFSGSGSGTDYSLTISNLEQEDIATYFCQQGNTLPYTFGGGTKLEITGSTSGSGKPGSGEGSTKGEVKLQESGPGLVAPSQSLSVTCTVSGVSLPDYGVSWIRQPPRKGLEWLGVIWGSETTYYNSALKSRLTIIKDNSKSQVFLKMNSLQTDDTAIYYCAKHYYYGGSYAMDYWGQGTSVTVSSIEVMYPPPYLDNEKSNGTIIHVKGKHLCPSPLFPGPSKPFWVLVVVGGVLACYSLLVTVAFIIFWVKRGRKKLLYIFKQPFMRPVQTTQEEDGCSCRFPEEEEGGCELRVKFSRSADAPAYQQGQNQLYNELNLGRREEYDVLDKRRGRDPEMGGKPRRKNPQEGLYNELQKDKMAEAYSEIGMKGERRRGKGHDGLYQGLSTATKDTYDALHMQALPPRRAKRSGSGEGRGSLLTCGDVEENPGPMDMRVPAQLLGLLLLWLRGARCEFKPLPEVTDEYAAAESKYGPPCPPCPMFWVLVVVGGVLACYSLLVTVAFIIFWVRSKRSRLLHSDYMNMTPRRPGPTRKHYQPYAPPRDFAAYRSRVKFSRSADAPAYQQGQNQLYNELNLGRREEYDVLDKRRGRDPEMGGKPRRKNPQEGLYNELQKDKMAEAYSEIGMKGERRRGKGHDGLYQGLSTATKDTYDALHMQALPPR

SEQ ID NO: 87 - protein, 887 aa, synthetic construct
  source 1..887: note = chimeric antigen receptor and switchable chimeric antigen receptor
MDMRVPAQLLGLLLLWLRGARCEFKPLPEVTDEYAAAESKYGPPCPPCPDIYIWAPLAGTCGVLLLSLVITLYCRSKRSRLLHSDYMNMTPRRPGPTRKHYQPYAPPRDFAAYRSRVKFSRSADAPAYQQGQNQLYNELNLGRREEYDVLDKRRGRDPEMGGKPRRKNPQEGLYNELQKDKMAEAYSEIGMKGERRRGKGHDGLYQGLSTATKDTYDALHMQALPPRGSGSSGEGRGSLLTCGDVEENPGPPVATMALPVTALLLPLALLLHAARPQVQLVESGGGLVQPGGSLRLSCAASGRTFSNYNMGWFRQAPGQGLEFVAAIDWSGGSPYYAASVRGRFTISRDNSKNTLYLQMNSLRAEDTAVYYCAAPLSYGSTWLADYWGQGTLVTVSSGGGGSGGGGSGGGGSGGGGSGGGGSDIQMTQTTSSLSASLGDRVTISCRASQDISKYLNWYQQKPDGTVKLLIYHTSRLHSGVPSRFSGSGSGTDYSLTISNLEQEDIATYFCQQGNTLPYTFGGGTKLEITGSTSGSGKPGSGEGSTKGEVKLQESGPGLVAPSQSLSVTCTVSGVSLPDYGVSWIRQPPRKGLEWLGVIWGSETTYYNSALKSRLTIIKDNSKSQVFLKMNSLQTDDTAIYYCAKHYYYGGSYAMDYWGQGTSVTVSSIEVMYPPPYLDNEKSNGTIIHVKGKHLCPSPLFPGPSKPFWVLVVVGGVLACYSLLVTVAFIIFWVKRGRKKLLYIFKQPFMRPVQTTQEEDGCSCRFPEEEEGGCELRVKFSRSADAPAYQQGQNQLYNELNLGRREEYDVLDKRRGRDPEMGGKPRRKNPQEGLYNELQKDKMAEAYSEIGMKGERRRGKGHDGLYQGLSTATKDTYDALHMQALPPR

SEQ ID NO: 88 - protein, 888 aa, synthetic construct
  source 1..888: note = chimeric antigen receptor and switchable chimeric antigen receptor
MALPVTALLLPLALLLHAARPQVQLVESGGGLVQPGGSLRLSCAASGRTFSNYNMGWFRQAPGQGLEFVAAIDWSGGSPYYAASVRGRFTISRDNSKNTLYLQMNSLRAEDTAVYYCAAPLSYGSTWLADYWGQGTLVTVSSGGGGSGGGGSGGGGSGGGGSGGGGSDIQMTQTTSSLSASLGDRVTISCRASQDISKYLNWYQQKPDGTVKLLIYHTSRLHSGVPSRFSGSGSGTDYSLTISNLEQEDIATYFCQQGNTLPYTFGGGTKLEITGSTSGSGKPGSGEGSTKGEVKLQESGPGLVAPSQSLSVTCTVSGVSLPDYGVSWIRQPPRKGLEWLGVIWGSETTYYNSALKSRLTIIKDNSKSQVFLKMNSLQTDDTAIYYCAKHYYYGGSYAMDYWGQGTSVTVSSIEVMYPPPYLDNEKSNGTIIHVKGKHLCPSPLFPGPSKPFWVLVVVGGVLACYSLLVTVAFIIFWVRSKRSRLLHSDYMNMTPRRPGPTRKHYQPYAPPRDFAAYRSRVKFSRSADAPAYQQGQNQLYNELNLGRREEYDVLDKRRGRDPEMGGKPRRKNPQEGLYNELQKDKMAEAYSEIGMKGERRRGKGHDGLYQGLSTATKDTYDALHMQALPPRRAKRSGSGEGRGSLLTCGDVEENPGPMDMRVPAQLLGLLLLWLRGARCEFKPLPEVTDEYAAAESKYGPPCPPCPMFWVLVVVGGVLACYSLLVTVAFIIFWVKRGRKKLLYIFKQPFMRPVQTTQEEDGCSCRFPEEEEGGCELRVKFSRSADAPAYQQGQNQLYNELNLGRREEYDVLDKRRGRDPEMGGKPRRKNPQEGLYNELQKDKMAEAYSEIGMKGERRRGKGHDGLYQGLSTATKDTYDALHMQALPPR

SEQ ID NO: 89 - protein, 887 aa, synthetic construct
  source 1..887: note = chimeric antigen receptor and switchable chimeric antigen receptor
MDMRVPAQLLGLLLLWLRGARCEFKPLPEVTDEYAAAESKYGPPCPPCPDIYIWAPLAGTCGVLLLSLVITLYCKRGRKKLLYIFKQPFMRPVQTTQEEDGCSCRFPEEEEGGCELRVKFSRSADAPAYQQGQNQLYNELNLGRREEYDVLDKRRGRDPEMGGKPRRKNPQEGLYNELQKDKMAEAYSEIGMKGERRRGKGHDGLYQGLSTATKDTYDALHMQALPPRGSGSSGEGRGSLLTCGDVEENPGPPVATMALPVTALLLPLALLLHAARPQVQLVESGGGLVQPGGSLRLSCAASGRTFSNYNMGWFRQAPGQGLEFVAAIDWSGGSPYYAASVRGRFTISRDNSKNTLYLQMNSLRAEDTAVYYCAAPLSYGSTWLADYWGQGTLVTVSSGGGGSGGGGSGGGGSGGGGSGGGGSDIQMTQTTSSLSASLGDRVTISCRASQDISKYLNWYQQKPDGTVKLLIYHTSRLHSGVPSRFSGSGSGTDYSLTISNLEQEDIATYFCQQGNTLPYTFGGGTKLEITGSTSGSGKPGSGEGSTKGEVKLQESGPGLVAPSQSLSVTCTVSGVSLPDYGVSWIRQPPRKGLEWLGVIWGSETTYYNSALKSRLTIIKDNSKSQVFLKMNSLQTDDTAIYYCAKHYYYGGSYAMDYWGQGTSVTVSSIEVMYPPPYLDNEKSNGTIIHVKGKHLCPSPLFPGPSKPFWVLVVVGGVLACYSLLVTVAFIIFWVRSKRSRLLHSDYMNMTPRRPGPTRKHYQPYAPPRDFAAYRSRVKFSRSADAPAYQQGQNQLYNELNLGRREEYDVLDKRRGRDPEMGGKPRRKNPQEGLYNELQKDKMAEAYSEIGMKGERRRGKGHDGLYQGLSTATKDTYDALHMQALPPR

SEQ ID NO: 90 - protein, 914 aa, synthetic construct
  source 1..914: note = chimeric antigen receptor and switchable chimeric antigen receptor
MALPVTALLLPLALLLHAARPQVQLVESGGGLVQPGGSLRLSCAASGRTFSNYNMGWFRQAPGQGLEFVAAIDWSGGSPYYAASVRGRFTISRDNSKNTLYLQMNSLRAEDTAVYYCAAPLSYGSTWLADYWGQGTLVTVSSGGGGSGGGGSGGGGSGGGGSGGGGSDIQMTQTTSSLSASLGDRVTISCRASQDISKYLNWYQQKPDGTVKLLIYHTSRLHSGVPSRFSGSGSGTDYSLTISNLEQEDIATYFCQQGNTLPYTFGGGTKLEITGSTSGSGKPGSGEGSTKGEVKLQESGPGLVAPSQSLSVTCTVSGVSLPDYGVSWIRQPPRKGLEWLGVIWGSETTYYNSALKSRLTIIKDNSKSQVFLKMNSLQTDDTAIYYCAKHYYYGGSYAMDYWGQGTSVTVSSIEVMYPPPYLDNEKSNGTIIHVKGKHLCPSPLFPGPSKPFWVLVVVGGVLACYSLLVTVAFIIFWVRSKRSRLLHSDYMNMTPRRPGPTRKHYQPYAPPRDFAAYRSRVKFSRSADAPAYQQGQNQLYNELNLGRREEYDVLDKRRGRDPEMGGKPRRKNPQEGLYNELQKDKMAEAYSEIGMKGERRRGKGHDGLYQGLSTATKDTYDALHMQALPPRRAKRSGSGEGRGSLLTCGDVEENPGPMDMRVPAQLLGLLLLWLRGARCEFKPLPEVTDEYAAAIEVMYPPPYLDNEKSNGTIIHVKGKHLCPSPLFPGPSKPFWVLVVVGGVLACYSLLVTVAFIIFWVKRGRKKLLYIFKQPFMRPVQTTQEEDGCSCRFPEEEEGGCELRVKFSRSADAPAYQQGQNQLYNELNLGRREEYDVLDKRRGRDPEMGGKPRRKNPQEGLYNELQKDKMAEAYSEIGMKGERRRGKGHDGLYQGLSTATKDTYDALHMQALPPR

SEQ ID NO: 91 - protein, 915 aa, synthetic construct
  source 1..915: note = chimeric antigen receptor and switchable chimeric antigen receptor
MALPVTALLLPLALLLHAARPQVQLVESGGGLVQPGGSLRLSCAASGRTFSNYNMGWFRQAPGQGLEFVAAIDWSGGSPYYAASVRGRFTISRDNSKNTLYLQMNSLRAEDTAVYYCAAPLSYGSTWLADYWGQGTLVTVSSGGGGSGGGGSGGGGSGGGGSGGGGSDIQMTQTTSSLSASLGDRVTISCRASQDISKYLNWYQQKPDGTVKLLIYHTSRLHSGVPSRFSGSGSGTDYSLTISNLEQEDIATYFCQQGNTLPYTFGGGTKLEITGSTSGSGKPGSGEGSTKGEVKLQESGPGLVAPSQSLSVTCTVSGVSLPDYGVSWIRQPPRKGLEWLGVIWGSETTYYNSALKSRLTIIKDNSKSQVFLKMNSLQTDDTAIYYCAKHYYYGGSYAMDYWGQGTSVTVSSAAAIEVMYPPPYLDNEKSNGTIIHVKGKHLCPSPLFPGPSKPFWVLVVVGGVLACYSLLVTVAFIIFWVRSKRSRLLHSDYMNMTPRRPGPTRKHYQPYAPPRDFAAYRSRVKFSRSADAPAYQQGQNQLYNELNLGRREEYDVLDKRRGRDPEMGGKPRRKNPQEGLYNELQKDKMAEAYSEIGMKGERRRGKGHDGLYQGLSTATKDTYDALHMQALPPRRAKRSGSGEGRGSLLTCGDVEENPGPMDMRVPAQLLGLLLLWLRGARCEFKPLPEVTDEYDIEVMYPPPYLDNEKSNGTIIHVKGKHLCPSPLFPGPSKPFWVLVVVGGVLACYSLLVTVAFIIFWVKRGRKKLLYIFKQPFMRPVQTTQEEDGCSCRFPEEEEGGCELRVKFSRSADAPAYQQGQNQLYNELNLGRREEYDVLDKRRGRDPEMGGKPRRKNPQEGLYNELQKDKMAEAYSEIGMKGERRRGKGHDGLYQGLSTATKDTYDALHMQALPPR

SEQ ID NO: 92 - protein, 884 aa, synthetic construct
  source 1..884: note = chimeric antigen receptor and switchable chimeric antigen receptor
MALPVTALLLPLALLLHAARPQVQLVESGGGLVQPGGSLRLSCAASGRTFSNYNMGWFRQAPGQGLEFVAAIDWSGGSPYYAASVRGRFTISRDNSKNTLYLQMNSLRAEDTAVYYCAAPLSYGSTWLADYWGQGTLVTVSSGGGGSGGGGSGGGGSGGGGSGGGGSDIQMTQTTSSLSASLGDRVTISCRASQDISKYLNWYQQKPDGTVKLLIYHTSRLHSGVPSRFSGSGSGTDYSLTISNLEQEDIATYFCQQGNTLPYTFGGGTKLEITGSTSGSGKPGSGEGSTKGEVKLQESGPGLVAPSQSLSVTCTVSGVSLPDYGVSWIRQPPRKGLEWLGVIWGSETTYYNSALKSRLTIIKDNSKSQVFLKMNSLQTDDTAIYYCAKHYYYGGSYAMDYWGQGTSVTVSSIEVMYPPPYLDNEKSNGTIIHVKGKHLCPSPLFPGPSKPFWVLVVVGGVLACYSLLVTVAFIIFWVRSKRSRLLHSDYMNMTPRRPGPTRKHYQPYAPPRDFAAYRSRVKFSRSADAPAYQQGQNQLYNELNLGRREEYDVLDKRRGRDPEMGGKPRRKNPQEGLYNELQKDKMAEAYSEIGMKGERRRGKGHDGLYQGLSTATKDTYDALHMQALPPRRAKRSGSGEGRGSLLTCGDVEENPGPMDMRVPAQLLGLLLLWLRGARCEFKPLPEVTDEYAAAESKYGPPCPPCPIYIWAPLAGTCGVLLLSLVITLYCKRGRKKLLYIFKQPFMRPVQTTQEEDGCSCRFPEEEEGGCELRVKFSRSADAPAYQQGQNQLYNELNLGRREEYDVLDKRRGRDPEMGGKPRRKNPQEGLYNELQKDKMAEAYSEIGMKGERRRGKGHDGLYQGLSTATKDTYDALHMQALPPR

SEQ ID NO: 93 - DNA, 2667 bp, synthetic construct
  source 1..2667: mol_type = other DNA; note = chimeric antigen receptor and switchable chimeric antigen receptor
atggcccttccagtgaccgccctgctgctgccactggctctgctgctgcacgccgctagacctcaggtgcagctggtggaaagcggcgggggcctggtgcagcctggcggcagcctgagactgtcttgcgccgctagcggaagaacttttagcaactacaacatgggctggtttagacaggcccccggccagggcctggagttcgtggctgccatcgactggagcggcggaagcccctattacgccgcctccgtgcggggcagattcaccatcagccgggacaattctaagaataccctgtatctgcaaatgaacagcctgagagccgaagatacagccgtgtactactgcgccgcccctctgagctacggaagcacatggctggccgactactggggacaaggaaccctggtaaccgtctcaagcggcggtggaggatcaggaggtggtggttcaggaggtggaggttctgggggaggcggatctgggggaggaggcagcgacatccagatgacacagacaacctccagcctgagcgccagcctgggcgacagagtgaccatcagctgtagagcctctcaggacatcagcaagtacctgaactggtatcagcagaaacctgatggcaccgtgaagctgctgatctaccacacatctaggctgcactctggagtccccagccggtttagcggaagcgggtcaggcacagactatagcctgaccatctccaatctggaacaggaggacatcgccacctacttctgccagcagggcaacaccctgccttatacattcggtggcggcaccaagctggaaatcaccggcagcacctctggctctggcaagcccggaagcggcgagggctccaccaagggagaggtgaagctgcaggagtccggacctgggctggtggctccaagccagagcctgagcgtgacctgcaccgtgtccggagtgagcctgcctgattacggcgtgtcttggatcagacagcctcctagaaagggactggaatggctgggcgtgatctggggtagcgagacaacatactacaacagcgccctgaagagcagactgacaatcatcaaggacaacagcaaaagccaggtgttcctaaaaatgaactccctgcagaccgacgacaccgccatctactactgtgcgaaacactactactacggcggctcctacgccatggactattggggccagggcaccagcgtgacagtgagcagcatcgaggtgatgtacccccctccttacctggacaacgagaagtccaacggcaccattatccacgtgaaaggcaagcacctgtgccccagccctctgttccccggcccttctaaaccgttctgggttctggtggtcgtgggcggcgtactggcttgctactctctgctggtcacagtggctttcatcatcttctgggtgaaaagaggcagaaagaaactgctgtacatctttaagcagccattcatgcggccagtgcagaccacccaggaggaggacggctgctcttgtcgctttcccgaggaggaggagggcggatgtgagctgagggtgaagtttagcagatccgctgatgcccctgcctatcagcagggacagaaccagctgtacaacgagctgaacctggggagaagagaagagtacgatgtgctggacaagcggagaggcagagatcctgagatgggcggcaagcccagacggaagaatcctcaagagggcctgtacaatgaactgcagaaagacaagatggccgaggcctacagcgagatcggaatgaagggcgagcgcagaagaggcaagggacacgatggactgtaccagggcctgagcaccgccaccaaggatacctatgatgccctgcacatgcaggccctgcctccaagaagagcaaagagatccggaagcggcgaaggcagaggatcactgcttacatgcggcgacgtggaagagaaccctggacctatggacatgagagtgccagctcagctgctgggcctgctgctgctgtggctgagaggcgccagatgcgagttcaagcctctgcctgaagtgaccgacgagtacgccgccgctgagtctaagtacggccctccttgtcctccttgccctatgttttgggtgctggttgtggttggaggcgtgctcgcttgttactccctcctggtgacagtcgcttttatcattttttgggtgcgcagcaagaggtccagactgctgcactctgactacatgaacatgactcccaggaggccaggccctactagaaaacactaccagccctacgctcctcctagagacttcgccgcctacaggtccagggtcaagttttccagaagcgctgacgctcccgcttaccagcagggccaaaatcagctctataacgaactgaatctcggcaggcgcgaggaatatgacgtgctggataagaggcggggacgcgaccctgaaatgggaggaaagcctcggcggaaaaacccacaagaaggactttacaacgaactccaaaaggataagatggctgaagcctactctgagattggcatgaaaggagaacgtcggagaggaaaaggccacgacggactctatcagggactgtctacagccacaaaagacacatacgacgcactccatatgcaggctctcccacctagataa

SEQ ID NO: 94 - DNA, 2664 bp, synthetic construct
  source 1..2664: mol_type = other DNA; note = chimeric antigen receptor and switchable chimeric antigen receptor
atggatatgagggtgccagcccagctgctgggcctgctgctgctgtggctgagaggagccaggtgtgaatttaagcccctgcctgaggtgactgacgagtacgccgcagctgagtccaagtacggcccaccctgcccaccctgcccagacatctacatttgggcccctctggccggaacatgcggagtgctgcttctgtcccttgtaatcaccctttattgtcgatccaagagatcacgactgctgcattctgattacatgaatatgactcctagacggccagggcccacaaggaagcactaccagccttatgcccctcctagagatttcgccgcctatagaagtagggtgaagtttagcagatccgctgatgcccctgcctatcagcagggacagaaccagctgtacaacgagctgaacctggggagaagagaagagtacgatgtgctggacaagcggagaggcagagatcctgagatgggcggcaagcccagacggaagaatcctcaagagggcctgtacaatgaactgcagaaagacaagatggccgaggcctacagcgagatcggaatgaagggcgagcgcagaagaggcaagggacacgatggactgtaccagggcctgagcaccgccaccaaggatacctatgatgccctgcacatgcaggcactgcctccaagaggatctggctcgagcggcgaaggcagaggatcactgcttacatgcggcgacgtggaagagaaccctggacctcctgtggccaccatggccctgccagtgaccgccctgctgctgcccctggcactgctgctgcacgcagccagaccccaagtgcagctggtggagtcaggcggcgggctagtgcagccaggaggctccctgagactgtcttgcgctgcaagcggcagaaccttctcaaactacaatatggggtggttcaggcaggcccccgggcagggcctggagttcgtggccgctatcgactggagtgggggctccccctactatgcagctagcgtgagaggcagatttaccatctccagagacaactccaagaacactctgtacctccagatgaatagtctgagagccgaagatacagccgtgtactactgtgccgcccccctgagctacggcagcacctggctggctgattactggggtcagggaacactggttacagtgtcatccggaggaggtggtagtggaggcggaggcagtggtggaggcggtagcgggggaggcggatctgggggaggaggcagcgacatccagatgacccagaccacctcctctctgagcgcttcactcggagaccgggtgacaatcagctgtagagcctcccaggatatctctaagtatctgaactggtaccagcagaagccagatggcacagtgaagctgctgatctatcataccagcaggctgcactccggagtgccttccaggttttccggcagcggatccggcaccgattatagcctgaccatctccaatctggagcaggaggacatagcaacctacttttgccagcagggcaataccctgccctacacctttgggggaggaaccaaactcgaaatcaccggctctacttctggaagcggcaagcccggatcaggcgaaggctcaaccaagggcgaggtgaaactgcaggagagcggcccaggactggtcgccccatcacagtccctgtcagtgacctgcaccgttagcggggtgtccctgcctgactacggggtgagctggatcaggcagcctcctcggaagggcctggagtggctgggggtgatctggggctccgagaccacctattataactccgccctgaagtcccggctgaccatcattaaagataacagcaagagccaggtgttcctgaagatgaactcactgcagacagacgacaccgctatctattattgcgccaagcattactactacggcggatcatacgccatggactattggggccagggcacttctgtgaccgtgtcttctatcgaggtgatgtaccccccaccatatctggataacgagaaatccaatggcaccatcattcacgtgaagggcaagcacctgtgtccatctcctctgttccctggcccaagcaagcccttctgggtgctggtggtcgtggggggcgtgctggcctgctactctctgctggtgactgtggcattcatcatcttctgggtgaagcggggcaggaagaaactgctgtacatcttcaagcagccattcatgcggcccgtgcagaccacccaggaagaggatgggtgctcatgccggttccctgaggaggaggagggggggtgcgagctgagggtcaagttttccagaagcgctgacgctcccgcttaccagcagggccaaaatcagctctataacgaactgaatctcggcaggcgcgaggaatatgacgtgctggataagaggcggggacgcgaccctgaaatgggaggaaagcctcggcggaaaaacccacaagaaggactttacaacgaactccaaaaggataagatggctgaagcctactctgagattggcatgaaaggagaacgtcggagaggaaaaggccacgacggactctatcagggactgtctacagccacaaaagacacatacgacgcactccatatgcaggctctcccacctagataa

SEQ ID NO: 95 - DNA, 2667 bp, synthetic construct
  source 1..2667: mol_type = other DNA; note = chimeric antigen receptor and switchable chimeric antigen receptor
atggccctgccagtgaccgccctgctgctgcccctggcactgctgctgcacgcagccagaccccaagtgcagctggtggagtcaggcggcgggctagtgcagccaggaggctccctgagactgtcttgcgctgcaagcggcagaaccttctcaaactacaatatggggtggttcaggcaggcccccgggcagggcctggagttcgtggccgctatcgactggagtgggggctccccctactatgcagctagcgtgagaggcagatttaccatctccagagacaactccaagaacactctgtacctccagatgaatagtctgagagccgaagatacagccgtgtactactgtgccgcccccctgagctacggcagcacctggctggctgattactggggacagggtacactggttacagtatcatctggcggtggaggatcaggaggtggtggttcaggaggtggaggttctgggggaggcggatctgggggaggaggcagcgacatccagatgacccagaccacctcctctctgagcgcttcactcggagaccgggtgacaatcagctgtagagcctcccaggatatctctaagtatctgaactggtaccagcagaagccagatggcacagtgaagctgctgatctatcataccagcaggctgcactccggagtgccttccaggttttccggcagcggatccggcaccgattatagcctgaccatctccaatctggagcaggaggacatagcaacctacttttgccagcagggcaataccctgccctacacctttgggggaggaaccaaactcgaaatcaccggctctacttctggaagcggcaagcccggatcaggcgaaggctcaaccaagggcgaggtgaaactgcaggagagcggcccaggactggtcgccccatcacagtccctgtcagtgacctgcaccgttagcggggtgtccctgcctgactacggggtgagctggatcaggcagcctcctcggaagggcctggagtggctgggggtgatctggggctccgagaccacctattataactccgccctgaagtcccggctgaccatcattaaagataacagcaagagccaggtgttcctgaagatgaactcactgcagacagacgacaccgctatctattattgcgccaagcattactactacggcggatcatacgccatggactattggggccagggcacttctgtgaccgtgtcttctatcgaggtgatgtaccccccaccatatctggataacgagaaatccaatggcaccatcattcacgtgaagggcaagcacctgtgtccatctcctctgttccctggcccaagcaagcccttctgggtgctggtggtcgtggggggcgtgctggcctgctactctctgctggtgactgtggcattcatcatcttctgggtgagatccaaaaggtctcgcctgctgcacagcgactatatgaatatgacccctcgcaggcctggccctacacgcaagcactatcagccttacgccccccctcgggactttgctgcgtatcggagtagggtgaagtttagcagatccgctgatgcccctgcctatcagcagggacagaaccagctgtacaacgagctgaacctggggagaagagaagagtacgatgtgctggacaagcggagaggcagagatcctgagatgggcggcaagcccagacggaagaatcctcaagagggcctgtacaatgaactgcagaaagacaagatggccgaggcctacagcgagatcggaatgaagggcgagcgcagaagaggcaagggacacgatggactgtaccagggcctgagcaccgccaccaaggatacctatgatgccctgcacatgcaggccctgcctccaagaagagcaaagagatccggaagcggcgaaggcagaggatcactgcttacatgcggcgacgtggaagagaaccctggacctatggacatgagagtgccagctcagctgctgggcctgctgctgctgtggctgagaggcgccagatgcgagttcaagcctctgcctgaagtgaccgacgagtacgccgccgctgagtctaagtacggccctccttgtcctccttgccctatgttttgggtcctggttgtggttggaggcgtgctcgcttgttactccctcctggtgacagtcgcttttatcattttttgggtgaagaggggccgcaagaagctgctgtatatctttaagcagccatttatgcggcccgtgcagaccacccaagaagaggacggatgtagctgcagatttcctgaggaagaagagggcggctgtgaactgagggtcaagttttccagaagcgctgacgctcccgcttaccagcagggccaaaatcagctctataacgaactgaatctcggcaggcgcgaggaatatgacgtgctggataagaggcggggacgcgaccctgaaatgggaggaaagcctcggcggaaaaacccacaagaaggactttacaacgaactccaaaaggataagatggctgaagcctactctgagattggcatgaaaggagaacgtcggagaggaaaaggccacgacggactctatcagggactgtctacagccacaaaagacacatacgacgcactccatatgcaggctctcccacctagataa

SEQ ID NO: 96 - DNA, 2664 bp, synthetic construct
  source 1..2664: mol_type = other DNA; note = chimeric antigen receptor and switchable chimeric antigen receptor
atggatatgagagtgccagcccagctgctgggcctgctgctgctgtggctgagaggcgccagatgcgagttcaagcctctgccagaggtgactgatgagtacgccgctgcagaatcaaagtacggccctccttgtccaccctgtccagacatctacatttgggcccccctggccgggacatgcggcgtgctcctgctgtctctggtgatcaccctgtactgtaaaagaggcagaaagaaactgctgtacatctttaagcagccattcatgcggccagtgcagaccacccaggaggaggacggctgctcttgtcgctttcccgaggaggaggagggcggatgtgagctgagggtgaagtttagcagatccgctgatgcccctgcctatcagcagggacagaaccagctgtacaacgagctgaacctggggagaagagaagagtacgatgtgctggacaagcggagaggcagagatcctgagatgggcggcaagcccagacggaagaatcctcaagagggcctgtacaatgaactgcagaaagacaagatggccgaggcctacagcgagatcggaatgaagggcgagcgcagaagaggcaagggacacgatggactgtaccagggcctgagcaccgccaccaaggatacctatgatgccctgcacatgcaggcactgcctccaagaggatctggctcgagcggcgaaggcagaggatcactgcttacatgcggcgacgtggaagagaaccctggacctcctgtggccaccatggccctgccagtgaccgccctgctgctgcccctggcactgctgctgcacgcagccagaccccaagtgcagctggtggagtcaggcggcgggctagtgcagccaggaggctccctgagactgtcttgcgctgcaagcggcagaaccttctcaaactacaatatggggtggttcaggcaggcccccgggcagggcctggagttcgtggccgctatcgactggagtgggggctccccctactatgcagctagcgtgagaggcagatttaccatctccagagacaactccaagaacactctgtacctccagatgaatagtctgagagccgaagatacagccgtgtactactgtgccgcccccctgagctacggcagcacctggctggctgattactggggacagggtacactggttacagtatcatctggcggtggaggatcaggaggtggtggttcaggaggtggaggttctgggggaggcggatctgggggaggaggcagcgacatccagatgacccagaccacctcctctctgagcgcttcactcggagaccgggtgacaatcagctgtagagcctcccaggatatctctaagtatctgaactggtaccagcagaagccagatggcacagtgaagctgctgatctatcataccagcaggctgcactccggagtgccttccaggttttccggcagcggatccggcaccgattatagcctgaccatctccaatctggagcaggaggacatagcaacctacttttgccagcagggcaataccctgccctacacctttgggggaggaaccaaactcgaaatcaccggctctacttctggaagcggcaagcccggatcaggcgaaggctcaaccaagggcgaggtgaaactgcaggagagcggcccaggactggtcgccccatcacagtccctgtcagtgacctgcaccgttagcggggtgtccctgcctgactacggggtgagctggatcaggcagcctcctcggaagggcctggagtggctgggggtgatctggggctccgagaccacctattataactccgccctgaagtcccggctgaccatcattaaagataacagcaagagccaggtgttcctgaagatgaactcactgcagacagacgacaccgctatctattattgcgccaagcattactactacggcggatcatacgccatggactattggggccagggcacttctgtgaccgtgtcttctatcgaggtgatgtaccccccaccatatctggataacgagaaatccaatggcaccatcattcacgtgaagggcaagcacctgtgtccatctcctctgttccctggcccaagcaagcccttctgggtgctggtggtcgtggggggcgtgctggcctgctactctctgctggtgactgtggcattcatcatcttctgggtgagatccaaaaggtctcgcctgctgcacagcgactatatgaatatgacccctcgcaggcctggccctacacgcaagcactatcagccttacgccccccctcgggactttgctgcgtatcggagtagggtcaagttttccagaagcgctgacgctcccgcttaccagcagggccaaaatcagctctataacgaactgaatctcggcaggcgcgaggaatatgacgtgctggataagaggcggggacgcgaccctgaaatgggaggaaagcctcggcggaaaaacccacaagaaggactttacaacgaactccaaaaggataagatggctgaagcctactctgagattggcatgaaaggagaacgtcggagaggaaaaggccacgacggactctatcagggactgtctacagccacaaaagacacatacgacgcactccatatgcaggctctcccacctagataa

SEQ ID NO: 97 - DNA, 2745 bp, synthetic construct
  source 1..2745: mol_type = other DNA; note = chimeric antigen receptor and switchable chimeric antigen receptor
atggccctgccagtgaccgccctgctgctgcccctggcactgctgctgcacgcagccagaccccaagtgcagctggtggagtcaggcggcgggctagtgcagccaggaggctccctgagactgtcttgcgctgcaagcggcagaaccttctcaaactacaatatggggtggttcaggcaggcccccgggcagggcctggagttcgtggccgctatcgactggagtgggggctccccctactatgcagctagcgtgagaggcagatttaccatctccagagacaactccaagaacactctgtacctccagatgaatagtctgagagccgaagatacagccgtgtactactgtgccgcccccctgagctacggcagcacctggctggctgattactggggacagggtacactggttacagtatcatctggcggtggaggatcaggaggtggtggttcaggaggtggaggttctgggggaggcggatctgggggaggaggcagcgacatccagatgacccagaccacctcctctctgagcgcttcactcggagaccgggtgacaatcagctgtagagcctcccaggatatctctaagtatctgaactggtaccagcagaagccagatggcacagtgaagctgctgatctatcataccagcaggctgcactccggagtgccttccaggttttccggcagcggatccggcaccgattatagcctgaccatctccaatctggagcaggaggacatagcaacctacttttgccagcagggcaataccctgccctacacctttgggggaggaaccaaactcgaaatcaccggctctacttctggaagcggcaagcccggatcaggcgaaggctcaaccaagggcgaggtgaaactgcaggagagcggcccaggactggtcgccccatcacagtccctgtcagtgacctgcaccgttagcggggtgtccctgcctgactacggggtgagctggatcaggcagcctcctcggaagggcctggagtggctgggggtgatctggggctccgagaccacctattataactccgccctgaagtcccggctgaccatcattaaagataacagcaagagccaggtgttcctgaagatgaactcactgcagacagacgacaccgctatctattattgcgccaagcattactactacggcggatcatacgccatggactattggggccagggcacttctgtgaccgtgtcttctatcgaggtgatgtaccccccaccatatctggataacgagaaatccaatggcaccatcattcacgtgaagggcaagcacctgtgtccatctcctctgttccctggcccaagcaagcccttctgggtgctggtggtcgtggggggcgtgctggcctgctactctctgctggtgactgtggcattcatcatcttctgggtgagatccaaaaggtctcgcctgctgcacagcgactatatgaatatgacccctcgcaggcctggccctacacgcaagcactatcagccttacgccccccctcgggactttgctgcgtatcggagtagggtgaagtttagcagatccgctgatgcccctgcctatcagcagggacagaaccagctgtacaacgagctgaacctggggagaagagaagagtacgatgtgctggacaagcggagaggcagagatcctgagatgggcggcaagcccagacggaagaatcctcaagagggcctgtacaatgaactgcagaaagacaagatggccgaggcctacagcgagatcggaatgaagggcgagcgcagaagaggcaagggacacgatggactgtaccagggcctgagcaccgccaccaaggatacctatgatgccctgcacatgcaggccctgcctccaagaagagcaaagagatccggaagcggcgaaggcagaggatcactgcttacatgcggcgacgtggaagagaaccctggacctatggacatgagagtgccagctcagctgctgggcctgctgctgctgtggctgagaggcgccagatgcgagttcaagcctctgcctgaagtgaccgacgagtacgccgccgctattgaagtcatgtatccacctccctatctggacaatgaaaagtctaatggcacaatcatccacgtcaagggaaaacacctgtgccctagccccctgtttcctggcccctctaaacccttttgggtcctggttgtggttggaggcgtgctcgcttgttactccctcctggtgacagtcgcttttatcattttttgggtgaagaggggccgcaagaagctgctgtatatctttaagcagccatttatgcggcccgtgcagaccacccaagaagaggacggatgtagctgcagatttcctgaggaagaagagggcggctgtgaactgagggtcaagttttccagaagcgctgacgctcccgcttaccagcagggccaaaatcagctctataacgaactgaatctcggcaggcgcgaggaatatgacgtgctggataagaggcggggacgcgaccctgaaatgggaggaaagcctcggcggaaaaacccacaagaaggactttacaacgaactccaaaaggataagatggctgaagcctactctgagattggcatgaaaggagaacgtcggagaggaaaaggccacgacggactctatcagggactgtctacagccacaaaagacacatacgacgcactccatatgcaggctctcccacctagataa

SEQ ID NO: 98 - DNA, 2748 bp, synthetic construct
  source 1..2748: mol_type = other DNA; note = chimeric antigen receptor and switchable chimeric antigen receptor
atggcccttccagtgaccgccctgctgctgccactggctctgctgctgcacgccgctagacctcaggtgcagctggtggaaagcgggggaggcctggttcagcccggcggcagcctgagactgagctgcgccgctagcggcagaacattcagcaactacaacatgggctggttcagacaagcccctggccagggcctggaattcgtggccgctatcgactggtccggcggcagcccttactacgccgcctccgtgcggggcagattcaccatctctcgggataatagcaagaacaccctctacctgcagatgaatagcctgagagccgaggataccgccgtgtactactgtgccgctcctctgtcttacggcagcacctggctggcagattactggggccagggcaccctggtgacagtgtccagcggcggaggaggcagcggcggaggcggaagcggcggtggtggctctggaggcggcggctccggcggtggcggcagtgatatccagatgacccagaccacttccagcctgtctgcctccctgggcgacagggtgactatcagctgccgcgccagccaggatatttcaaaatacctgaattggtaccagcagaagcccgacggcacagtgaagctgctgatctaccacaccagtcgcctgcacagcggcgtgcccagcaggttcagcggcagcggatccggcacagactacagcctgaccatcagcaacctggagcaggaggatatcgcaacttatttttgccagcagggcaatacactgccttacaccttcggcggcggcaccaagctggaaatcaccggcagcacaagtggctccggcaaaccaggcagcggagagggcagcacaaagggcgaggtgaaactgcaggagagcggccccggcctggtggcccccagccagtctctgagcgtgacctgcaccgtgtccggcgtgtccctgcctgactacggggtgagctggatcaggcagccccccaggaaaggcttggaatggctgggcgtgatctggggcagcgagacaacctattataactctgccctgaagagcagactgaccatcatcaaagacaatagcaaaagccaggtgttcctgaagatgaattcactgcagactgacgatactgccatctattattgtgccaaacactactactatggcggatcctatgccatggattactggggccagggcacctcagtgaccgtgtcctcggccgctgctattgaagtgatgtatccacccccttacctggacaacgagaaatcaaacggcactattatccacgtgaagggaaagcacctgtgcccctcccctctgtttcccggcccaagtaagcccttttgggtgctggtggtggtcgggggcgtgctggcctgttattccctgctggtcacagtggctttcatcatcttctgggtgcgcagcaagaggtccagactgctgcactctgactacatgaacatgactcccaggaggccaggccctactagaaaacactaccagccctacgctcctcctagagacttcgccgcctacaggtccagggtcaagttttccagaagcgctgacgctcccgcttaccagcagggccaaaatcagctctataacgaactgaatctcggcaggcgcgaggaatatgacgtgctggataagaggcggggacgcgaccctgaaatgggaggaaagcctcggcggaaaaacccacaagaaggactttacaacgaactccaaaaggataagatggctgaagcctactctgagattggcatgaaaggagaacgtcggagaggaaaaggccacgacggactctatcagggactgtctacagccacaaaagacacatacgacgcactccatatgcaggctctcccacctagaagagcaaagagatccggaagcggcgaaggcagaggatcactgcttacatgcggcgacgtggaagagaaccctggacctatggatatgagagtgccagcccagctgctgggcctgctgctgctgtggctgagaggcgccagatgcgagttcaagcctctgccagaggtgactgatgagtacgacatcgaggtgatgtacccccctccttacctggacaacgagaagtccaacggcaccattatccacgtgaaaggcaagcacctgtgccccagccctctgttccccggcccttctaaaccgttctgggttctggtggtcgtgggcggcgtactggcttgctactctctgctggtcacagtggctttcatcatcttctgggtgaaaagaggcagaaagaaactgctgtacatctttaagcagccattcatgcggccagtgcagaccacccaggaggaggacggctgctcttgtcgctttcccgaggaggaggagggcggatgtgagctgagggtgaagtttagcagatccgctgatgcccctgcctatcagcagggacagaaccagctgtacaacgagctgaacctggggagaagagaagagtacgatgtgctggacaagcggagaggcagagatcctgagatgggcggcaagcccagacggaagaatcctcaagagggcctgtacaatgaactgcagaaagacaagatggccgaggcctacagcgagatcggaatgaagggcgagcgcagaagaggcaagggacacgatggactgtaccagggcctgagcaccgccaccaaggatacctatgatgccctgcacatgcaggccctgcctccaagataa

SEQ ID NO: 99 - DNA, 2655 bp, synthetic construct
  source 1..2655: mol_type = other DNA; note = chimeric antigen receptor and switchable chimeric antigen receptor
atggcccttccagtgaccgccctgctgctgccactggctctgctgctgcacgccgctagacctcaggtgcagctggtggaaagcgggggaggcctggttcagcccggcggcagcctgagactgagctgcgccgctagcggcagaacattcagcaactacaacatgggctggttcagacaagcccctggccagggcctggaattcgtggccgctatcgactggtccggcggcagcccttactacgccgcctccgtgcggggcagattcaccatctctcgggataatagcaagaacaccctctacctgcagatgaatagcctgagagccgaggataccgccgtgtactactgtgccgctcctctgtcttacggcagcacctggctggcagattactggggccagggcaccctggtgacagtgtccagcggcggaggaggcagcggcggaggcggaagcggcggtggtggctctggaggcggcggctccggcggtggcggcagtgatatccagatgacccagaccacttccagcctgtctgcctccctgggcgacagggtgactatcagctgccgcgccagccaggatatttcaaaatacctgaattggtaccagcagaagcccgacggcacagtgaagctgctgatctaccacaccagtcgcctgcacagcggcgtgcccagcaggttcagcggcagcggatccggcacagactacagcctgaccatcagcaacctggagcaggaggatatcgcaacttatttttgccagcagggcaatacactgccttacaccttcggcggcggcaccaagctggaaatcaccggcagcacaagtggctccggcaaaccaggcagcggagagggcagcacaaagggcgaggtgaaactgcaggagagcggccccggcctggtggcccccagccagtctctgagcgtgacctgcaccgtgtccggcgtgtccctgcctgactacggggtgagctggatcaggcagccccccaggaaaggcttggaatggctgggcgtgatctggggcagcgagacaacctattataactctgccctgaagagcagactgaccatcatcaaagacaatagcaaaagccaggtgttcctgaagatgaattcactgcagactgacgatactgccatctattattgtgccaaacactactactatggcggatcctatgccatggattactggggccagggcacctcagtgaccgtgtcctcgattgaagtgatgtatccacccccttacctggacaacgagaaatcaaacggcactattatccacgtgaagggaaagcacctgtgcccctcccctctgtttcccggcccaagtaagcccttttgggtgctggtggtggtcgggggcgtgctggcctgttattccctgctggtcacagtggctttcatcatcttctgggtgcgcagcaagaggtccagactgctgcactctgactacatgaacatgactcccaggaggccaggccctactagaaaacactaccagccctacgctcctcctagagacttcgccgcctacaggtccagggtcaagttttccagaagcgctgacgctcccgcttaccagcagggccaaaatcagctctataacgaactgaatctcggcaggcgcgaggaatatgacgtgctggataagaggcggggacgcgaccctgaaatgggaggaaagcctcggcggaaaaacccacaagaaggactttacaacgaactccaaaaggataagatggctgaagcctactctgagattggcatgaaaggagaacgtcggagaggaaaaggccacgacggactctatcagggactgtctacagccacaaaagacacatacgacgcactccatatgcaggctctcccacctagaagagcaaagagatccggaagcggcgaaggcagaggatcactgcttacatgcggcgacgtggaagagaaccctggacctatggatatgagagtgccagcccagctgctgggcctgctgctgctgtggctgagaggcgccagatgcgagttcaagcctctgccagaggtgactgatgagtacgcagccgctgaatcaaagtacggccctccttgtccaccctgtccaatctacatttgggcccccctggccgggacatgcggcgtgctcctgctgtctctggtgatcaccctgtactgtaaaagaggcagaaagaaactgctgtacatctttaagcagccattcatgcggccagtgcagaccacccaggaggaggacggctgctcttgtcgctttcccgaggaggaggagggcggatgtgagctgagggtgaagtttagcagatccgctgatgcccctgcctatcagcagggacagaaccagctgtacaacgagctgaacctggggagaagagaagagtacgatgtgctggacaagcggagaggcagagatcctgagatgggcggcaagcccagacggaagaatcctcaagagggcctgtacaatgaactgcagaaagacaagatggccgaggcctacagcgagatcggaatgaagggcgagcgcagaagaggcaagggacacgatggactgtaccagggcctgagcaccgccaccaaggatacctatgatgccctgcacatgcaggccctgcctccaagataa

SEQ ID NO: 100 - protein, 219 aa, synthetic construct
  source 1..219: note = targeting module chain
DIVMTQSPDSLAVSLGERATINCKSSQSLLNSRTPKNYLAWYQQKPGQPPKLLIYWASTRKSGVPDRFSGSGSGTDFTLTISSLQAEDVAVYYCKQSYNLLTFGGGTKVEIKRTVAAPSVFIFPPSDEQLKSGTASVVCLLNNFYPREAKVQWKVDNALQSGNSQESVTEQDSKDSTYSLSSTLTLSKADYEKHKVYACEVTHQGLSSPVTKSFNRGEC

SEQ ID NO: 101 - protein, 480 aa, synthetic construct
  source 1..480: note = targeting module chain
QVQLVESGGGLVQPGGSLRLSCVASGFTFSSNAMSWVRQAPGKGLEWVSAISGSGDYTHYSDSVKGRFTISRDNSKNTLYLQMNSLRAEDTAVYYCAKEVPGGPLVDFDSRGQGTLVTVSSGGGGSGGGGSQVQLVESGGGLVQPGGSLRLSCVASGFTFSSNAMSWVRQAPGKGLEWVSAISGSGDYTHYSDSVKGRFTISRDNSKNTLYLQMNSLRAEDTAVYYCAKEVPGGPLVDFDSRGQGTLVTVSSESKYGPPCPPCPAPEAAGGPSVFLFPPKPKDTLMISRTPEVTCVVVDVSQEDPEVQFNWYVDGVEVHNAKTKPREEQFNSTYRVVSVLTVLHQDWLNGKEYKCKVSNKGLPSSIEKTISKAKGQPREPQVYTLPPSQEEMTKNQVSLSCAVKGFYPSDIAVEWESNGQPENNYKTTPPVLDSDGSFFLVSRLTVDKSRWQEGNVFSCSVMHEALHNHYTQKSLSLSLG

SEQ ID NO: 102 - protein, 446 aa, synthetic construct
  source 1..446: note = targeting module chain
QVQLVQSGAEVKKPGASVKVSCKASGYTFTHYYIYWVRQAPGQGLEWMGGVNPSNGGTHFNEKFKSRVTMTRDTSISTAYMELSRLRSDDTAVYYCARSEYDYGLGFAYWGQGTLVTVSSASTKGPSVFPLAPCSRSTSESTAALGCLVKDYFPEPVTVSWNSGALTSGVHTFPAVLQSSGLYSLSSVVTVPSSSLGTKTYTCNVDHKPSNTKVDKRVESKYGPPCPPCPAPEAAGGPSVFLFPPKPKDTLMISRTPEVTCVVVDVSQEDPEVQFNWYVDGVEVHNAKTKPREEQFNSTYRVVSVLTVLQQDWLNGKEYKCKVSNKGLPSSIEKTISKAKGQPREPQVYTLPPSQEEMTKNQVSLWCLVKGFYPSDIAVEWESNGQPENNYKTTPPVLDSDGSFFLYSRLTVDKSRWQEGNVFSCSVMHEALHNHYTQKSLSLSLG